European Patent Specification EP 3 275 312 B1, published August 30, 2023. Title: Method of producing a transplanted fish. Applicant: National University Corporation Tokyo University of Marine Science and Technology. The sequence listing filed with the application follows.

SEQUENCE LISTING (6 sequences)

SEQ ID NO: 1 - DNA, 20 bp, Artificial Sequence
  forward primer_vasa
ctatttgttcctggctgtgg

SEQ ID NO: 2 - DNA, 23 bp, Artificial Sequence
  reverse primer_vasa
gcagactcttctaaccatgaagg

SEQ ID NO: 3 - DNA, 20 bp, Artificial Sequence
  forward primer_vasa of T.orientalis
ctaccagcattcacggtgac

SEQ ID NO: 4 - DNA, 20 bp, Artificial Sequence
  reverse primer_vasa of T.orientalis
gtagcaggtccgctgaacgc

SEQ ID NO: 5 - DNA, 20 bp, Artificial Sequence
  forward primer_gsdf
gctctcaacttgcaggctga

SEQ ID NO: 6 - DNA, 20 bp, Artificial Sequence
  reverse primer_gsdf
cccagcccagatctttcatg